European Patent Specification EP 3 503 920 B1, published May 8, 2024. Title: ANTI-CTLA4 ANTIBODIES. Applicant: Akeso Biopharma, Inc. Li, Baiyong Xia, Yu Wang, Zhongmin Zhang, Peng Pang, Xinghua. The sequence listing filed with the application follows.

SEQUENCE LISTING (36 sequences)

SEQ ID NO: 1 - protein, 364 aa, Artificial Sequence
  CTLA4-mFc fusion protein
AMHVAQPAVVLASSRGIASFVCEYASPGKATEVRVTVLRQADSQVTEVCAATYMMGNELTFLDDSICTGTSSGNQVNLTIQGLRAMDTGLYICKVELMYPPPYYLGIGNGTQIYVIDPEPCPDSDENLYFQGPRGPTIKPCPPCKCPAPNLLGGPSVFIFPPKIKDVLMISLSPIVTCVVVDVSEDDPDVQISWFVNNVEVHTAQTQTHREDYNSTLRVVSALPIQHQDWMSGKEFKCKVNNKDLPAPIERTISKPKGSVRAPQVYVLPPPEEEMTKKQVTLTCMVTDFMPEDIYVEWTNNGKTELNYKNTEPVLDSDGSYFMYSKLRVEKKNWVERNSYSCSVVHEGLHNHHTTKSFSRTPGK

SEQ ID NO: 2 - DNA, 1092 bp, Artificial Sequence
  CTLA4-mFC fusion
gcaatgcatgtcgcacagcctgcagtggtcctggcaagctccaggggaatcgctagcttcgtgtgcgaatacgcttccccaggcaaggcaaccgaggtccgggtgacagtcctgagacaggccgacagccaggtgacagaagtctgcgccgctacttatatgatgggcaacgagctgacctttctggacgatagcatttgtaccgggacatctagtggaaaccaagtgaatctgaccatccagggcctgcgcgctatggacacagggctgtacatttgtaaagtggagctgatgtatccccctccatactatctgggaatcggcaacgggacccagatctacgtgattgatcctgaaccatgccccgactccgatgagaatctgtatttccagggaccacgaggccccacaattaagccatgtcccccttgcaaatgtcctgcaccaaacctgctgggaggaccaagcgtgttcatctttccacccaagatcaaggacgtgctgatgatctcactgagccccattgtgacctgcgtggtcgtggacgtgagcgaggacgatcctgatgtgcagatcagttggttcgtcaacaatgtggaagtccacacagctcagactcagacccatagggaggattacaatagtactctgcgcgtcgtgtcagcactgcccattcagcaccaggactggatgagcggcaaggagttcaagtgcaaagtgaacaacaaggatctgcccgcacctatcgagagaactatttccaagcctaaagggtctgtgagggccccacaggtgtatgtcctgcctccacccgaggaagagatgactaagaaacaggtgacactgacttgtatggtcaccgacttcatgcccgaagatatctacgtggagtggactaacaatgggaagaccgaactgaactataaaaatacagagcctgtgctggactcagatggaagctactttatgtatagcaagctgcgagtggaaaagaaaaactgggtcgagcggaacagctactcttgtagtgtggtccacgaagggctgcataatcaccacaccactaaatcattctcccgaactccaggcaaa

SEQ ID NO: 3 - DNA, 372 bp, Mus musculus
caggtcaagctgcaggagtctggacctgagctggtgaagcctggagcttcaatgaagatatcctgcaaggcttctggttactcattcactggctacaccatgaactgggtgaagcagagccatggaaagaaccttgaatggattggacttattaatccttacaataatattactaactacaaccagaagttcatgggcaaggccacatttactgtagacaagtcatccagcacagcctacatggaactcctcagactgacatctgaagactctggagtctatttctgtgcaagactcgactataggtcttattggggccaagggactctggtcactgtctctgcagccaaaacgacacccccatctgtctat

SEQ ID NO: 4 - protein, 115 aa, Mus musculus
QVKLQESGPELVKPGASMKISCKASGYSFTGYTMNWVKQSHGKNLEWIGLINPYNNITNYNQKFMGKATFTVDKSSSTAYMELLRLTSEDSGVYFCARLDYRSYWGQGTLVTVSA

SEQ ID NO: 5 - DNA, 378 bp, Mus musculus
caggctgttgtgactcaggaatctgcactcaccacatcacctggtgaaacagtcacactcacttgtcgctcaagtactggggctgttacaactagtaactttgccaactgggtccaagaaaaaccagatcatttattcactagtctaataggtggtaccaacaaccgagctccaggtgttcctgccagattctcaggctccctgattggagacaaggctgccctcaccatcacaggggcacagactgaggatgaggcaatatatttctgtgctctatggtacagcaaccattgggtgttcggtggaggaaccaaactgactgtcctaggccagcccaagtcttcgccatcagtcaccctgtttcaagggcaattctgc

SEQ ID NO: 6 - protein, 126 aa, Mus musculus
QAVVTQESALTTSPGETVTLTCRSSTGAVTTSNFANWVQEKPDHLFTSLIGGTNNRAPGVPARFSGSLIGDKAALTITGAQTEDEAIYFCALWYSNHWVFGGGTKLTVLGQPKSSPSVTLFQGQFC

SEQ ID NO: 7 - DNA, 345 bp, Artificial Sequence
  humanized light chain variable region of 4G10H1L1
caggtgcagctggtggagtctggggccgagctggtgaagcccggcgcctccatgaagatctcttgcaaggccagcggatacagtttcactggctataccatgaactgggtcaaacaggctccaggacagggactggagtggatcgggctgattaatccttacaacaacatcaccaactacaaccagaagttcatgggaaaagcaacctttacagtggacaagagcatttccacagcctacatggaactgagccggctgacttcagacgatagcggggtctatttttgtgcaaggctggattatcgctcttactgggggcagggaactctggtcactgtctccgct

SEQ ID NO: 8 - protein, 115 aa, Artificial Sequence
  humanized heavy chain variable region of 4G10H1L1
QVQLVESGAELVKPGASMKISCKASGYSFTGYTMNWVKQAPGQGLEWIGLINPYNNITNYNQKFMGKATFTVDKSISTAYMELSRLTSDDSGVYFCARLDYRSYWGQGTLVTVSA

SEQ ID NO: 9 - DNA, 327 bp, Artificial Sequence
  humanized light chain variable region of 4G10H1L1
caggctgtcgtcactcaggaaccttcactgactgtgagcccaggaggaactgtcaccctgacatgcggaagctccaccggagcagtgaccacatccaacttcgccaattgggtccaggaaaagccaggccaggcatttcgatccctgatcggaggcacaaacaatcgggcttcttgggtgcccgcaagattctcaggaagcctgctggggggaaaagccgctctgaccattagtggcgctcagcctgaggacgaagccgagtacttctgcgctctgtggtatagcaaccactgggtgtttggcgggggaacaaagctgactgtgctg

SEQ ID NO: 10 - protein, 109 aa, Artificial Sequence
  humanized light chain variable region of 4G10H1L1
QAVVTQEPSLTVSPGGTVTLTCGSSTGAVTTSNFANWVQEKPGQAFRSLIGGTNNRASWVPARFSGSLLGGKAALTISGAQPEDEAEYFCALWYSNHWVFGGGTKLTVL

SEQ ID NO: 11 - DNA, 345 bp, Artificial Sequence
  humanized heavy chain variable region of 4G10H3L3
caggtgcagctggtcgagtctggggccgaagtgaagaaacccggcgcctcagtgaaggtcagctgcaaggccagcgggtacagtttcactggatataccatgaactgggtccgacaggcccctggccaggggctggagtggatcggcctgattaacccttacaacaacatcactaactacgcacagaagttccaggggagagtgacctttacagtggacaccagcatttccacagcctacatggaactgtcccggctgagatctgacgatacaggcgtgtacttctgcgctaggctggattaccgcagctattggggacagggcacactggtgactgtcagcgca

SEQ ID NO: 12 - protein, 115 aa, Artificial Sequence
  humanized heavy chain variable region of 4G10H3L3
QVQLVESGAEVKKPGASVKVSCKASGYSFTGYTMNWVRQAPGQGLEWIGLINPYNNITNYAQKFQGRVTFTVDTSISTAYMELSRLRSDDTGVYFCARLDYRSYWGQGTLVTVSA

SEQ ID NO: 13 - DNA, 327 bp, Artificial Sequence
  humanized light chain variable region of 4G10H3L3
caggctgtcgtcactcaggaaccttcactgaccgtgtctcctggcgggactgtcaccctgacatgcggcagctccacaggggccgtgaccacaagtaacttcccaaattgggtccagcagaagccaggacaggctccccggagtctgatcggaggcaccaacaacaaggccagctggacacccgcacggttcagcggcagcctgctgggcggcaaggccgctctgacaattagcggagcccagcctgaggacgaagccgagtactattgcgctctgtggtactccaaccactgggtgttcggcggcggcaccaagctgactgtgctg

SEQ ID NO: 14 - protein, 109 aa, Artificial Sequence
  humanized light chain variable region of 4G10H3L3
QAVVTQEPSLTVSPGGTVTLTCGSSTGAVTTSNFPNWVQQKPGQAPRSLIGGTNNKASWTPARFSGSLLGGKAALTISGAQPEDEAEYYCALWYSNHWVFGGGTKLTVL

SEQ ID NO: 15 - DNA, 345 bp, Artificial Sequence
  humanized heavy chain variable region 4G10H4
caggtgcagctggtcgagtctggggccgaagtgaagaaacccggcgcctcagtgaaggtcagctgcaaggccagcgggtacagtttcactggatataccatgaactgggtccgacaggcccctggccaggggctggagtggatcggcctgattaacccttacaacgacatcactaactacgcacagaagttccaggggagagtgacctttacagtggacaccagcatttccacagcctacatggaactgtcccggctgagatctgacgatacaggcgtgtacttctgcgctaggctggattaccgcagctattggggacagggcacactggtgactgtcagcgca

SEQ ID NO: 16 - protein, 115 aa, Artificial Sequence
  humanized heavy chain variable region 4G10H4
QVQLVESGAEVKKPGASVKVSCKASGYSFTGYTMNWVRQAPGQGLEWIGLINPYNDITNYAQKFQGRVTFTVDTSISTAYMELSRLRSDDTGVYFCARLDYRSYWGQGTLVTVSA

SEQ ID NO: 17 - DNA, 345 bp, Artificial Sequence
  humanized heavy chain variable region 4G10H5
caggtgcagctggtcgagtctggggccgaagtgaagaaacccggcgcctcagtgaaggtcagctgcaaggccagcgggtacagtttcactggatataccatgaactgggtccgacaggcccctggccaggggctggagtggatcggcctgattaacccttacaacaacatcgataactacgcacagaagttccaggggagagtgacctttacagtggacaccagcatttccacagcctacatggaactgtcccggctgagatctgacgatacaggcgtgtacttctgcgctaggctggattaccgcagctattggggacagggcacactggtgactgtcagcgca

SEQ ID NO: 18 - protein, 115 aa, Artificial Sequence
  humanized heavy chain variable region 4G10H5
QVQLVESGAEVKKPGASVKVSCKASGYSFTGYTMNWVRQAPGQGLEWIGLINPYNNIDNYAQKFQGRVTFTVDTSISTAYMELSRLRSDDTGVYFCARLDYRSYWGQGTLVTVSA

SEQ ID NO: 19 - protein, 115 aa, Artificial Sequence
  humanized 4G10 variable heavy chain region consensus sequence
  X (11)..(11): Val or Leu
  X (18)..(18): Val or Met
  X (20)..(20): Val or Ile
  X (34)..(34): Met or Val or Leu or Ile or Gly or Ala or Ser or Thr
  X (38)..(38): Arg or Lys
  X (56)..(56): Asn or Asp or Glu
  X (58)..(58): Thr or Asp or Glu or Gly or Ala
  X (61)..(61): Ala or Asn
  X (65)..(65): Gln or Met
  X (67)..(67): Arg or Lys
  X (68)..(68): Val or Ala
  X (74)..(74): Thr or Lys
  X (87)..(87): Arg or Thr
  X (91)..(91): Thr or Ser
QVQLVESGAEXKKPGASXKXSCKASGYSFTGYTXNWVXQAPGQGLEWIGLINPYNXIXNYXQKFXGXXTFTVDXSISTAYMELSRLXSDDXGVYFCARLDYRSYWGQGTLVTVSA

SEQ ID NO: 20 - protein, 109 aa, Artificial Sequence
  humanized 4G10 variable light chain region consensus sequence
  X (35)..(35): Pro or Ala
  X (40)..(40): Gln or Glu
  X (46)..(46): Pro or Phe
  X (56)..(56): Lys or Arg or any other amino acid except Met or Cys
  X (58)..(58): Ser or Pro
  X (60)..(60): Thr or Val
  X (89)..(89): Tyr or Phe
  X (93)..(93): Trp or any amino acid except Met or Cys
  X (98)..(98): Trp or any amino acid except Met or Cys
QAVVTQEPSLTVSPGGTVTLTCGSSTGAVTTSNFXNWVQXKPGQAXRSLIGGTNNXAXWXPARFSGSLLGGKAALTISGAQPEDEAEYXCALXYSNHXVFGGGTKLTVL

SEQ ID NO: 21 - protein, 5 aa, Artificial Sequence
  4G10 HCDR1 consensus
  X (4)..(4): Met or Val or Leu or Ile or Gly or Ala or Ser or Thr
GYTXN

SEQ ID NO: 22 - protein, 17 aa, Artificial Sequence
  4G10 HCDR2 consensus sequence
  X (7)..(7): Asn or Asp
  X (9)..(9): Thr or Asp or Glu or Gly or Ala
  X (12)..(12): Ala or Asn
  X (16)..(16): Gln or Met
LINPYNXIXNYXQKFXG

SEQ ID NO: 23 - protein, 6 aa, Artificial Sequence
  4G10 HCDR3 sequence
LDYRSY

SEQ ID NO: 24 - protein, 14 aa, Artificial Sequence
  4G10 LCDR1 consensus sequence
  X (13)..(13): Pro or Ala
GSSTGAVTTSNFXN

SEQ ID NO: 25 - protein, 7 aa, Artificial Sequence
  4G10 LCDR2 consensus sequence
  X (5)..(5): Lys or Arg or any amino acid except Met or Cys
  X (7)..(7): Ser or Pro
GTNNXAX

SEQ ID NO: 26 - protein, 8 aa, Artificial Sequence
  4G10 LCDR3 consensus sequence
  X (3)..(3): Trp or any amino acid except Met or Cys
  X (8)..(8): Trp or any amino acid except Met or Cys
ALXYSNHX

SEQ ID NO: 27 - protein, 8 aa, Artificial Sequence
  4G10 HCDR1 sequence
GYSFTGYT

SEQ ID NO: 28 - protein, 8 aa, Artificial Sequence
  4G10 HCDR2
  X (6)..(6): Asn or Asp or Glu
  X (8)..(8): Thr or Asp or Glu or Gly or Ala
INPYNXIX

SEQ ID NO: 29 - protein, 8 aa, Artificial Sequence
  4G10 HCDR3
ARLDYRSY

SEQ ID NO: 30 - protein, 9 aa, Artificial Sequence
  4G10 LCDR1
TGAVTTSNF

SEQ ID NO: 31 - protein, 3 aa, Artificial Sequence
  4G10 LCDR2
GTN

SEQ ID NO: 32 - protein, 9 aa, Artificial Sequence
  4G10 LCDR3
  X (3)..(3): Trp or any amino acid except Met or Cys
  X (8)..(8): Trp or any amino acid except Met or Cys
ALXYSNHXV

SEQ ID NO: 33 - protein, 330 aa, Artificial Sequence [sequence omitted]

SEQ ID NO: 34 - protein, 107 aa, Artificial Sequence [sequence omitted]

SEQ ID NO: 35 - protein, 443 aa, Artificial Sequence
  10D1 heavy chain
QVQLVESGGGVVQPGRSLRLSCAASGFTFSSYTMHWVRQAPGKGLEWVTFISYDGNNKYYADSVKGRFTISRDNSKNTLYLQMNSLRAEDTAIYYCARTGWLGPFDYWQGTLVTVSSASTKGPSVFPLAPSSKSTSGGTAALGCLVKDYFPEPVTVSWNSGALTSGVHTFPAVLQSSGLYSLSSVVTVPSSSLGTQTYICNVNHKPSNTKVDKKVEPKSCDKTHTCPPCPAPELLGPSVFLFPPPKDTLMISRTPEVTCVVVDVSHEDPEVKFNWYVDGVEVHNAKTKPREEQYNSTYRVVSVLTVLHQDWLNGKEYKCKVSNKALPAPIEKTISKAKGQPREPQVYTLPPSRDELTKNQVLTCLVKGFYPDIAVEWESNGQPENNYKTTPPVLDSDGSFFLYSKLTVDKSRWQQGNVFSCSVMHEALHNHYTQKSLSLSPGK

SEQ ID NO: 36 - protein, 214 aa, Artificial Sequence
  10D1 Light chain
EIVLTQSPGTLSLSPGERATLSCRASQSVGSSYLAWYQQKPGQAPRLLIYGAFSRATGIPDRFSGSGSGTDFTLTISRLEPEDFAVYYCQQYGSSPWTFGQGTKVEIKTVAAPSVFIFPPSDEQLKSGTASVVCLLNNFYPREAKVQWKVDNALQSGNSQESVTEQDSKDSTYSLSSTLTLSKADYEKHKVYACEVTHQGLSSPVTKSFNRGEC